European Patent Specification EP 3 960 195 B1, published January 8, 2025. Title: Treatment of DNA-damage and age-related diseases or disorders. Applicant: Centre National de la Recherche Scientifique Institut National de la Recherche Medicale College de France. The sequence listing filed with the application follows.

SEQUENCE LISTING (50 sequences)

SEQ ID NO: 1 - protein, 60 aa, artificial sequence
  synthetic polypeptide
RRRKRTAYTRYQLLELEKEFLFNRYLTRRRRIELAHSLNLTERHIKIWFQNRRMKWKKEN

SEQ ID NO: 2 - protein, 401 aa, Mus musculus
MEEQQPEPKSQRDSGLGAVAAAAPSGLSLSLSPGASGSSGSDGDSVPVSPQPAPPSPPAAPCLPPLAHHPHLPPHPPPPPPPPPPPPQHLAAPAHQPQPAAQLHRTTNFFIDNILRPDFGCKKEQPLPQLLVASAAAGGGAAAGGGSRVERDRGQTGAGRDPVHSLGTRASGAASLLCAPDANCGPPDGSQPATAVGAGASKAGNPAAAAAAAAAAAAAAVAAAAAAASKPSDSGGGSGGNAGSPGAQGAKFPEHNPAILLMGSANGGPVVKTDSQQPLVWPAWVYCTRYSDRPSSGPRTRKLKKKKNEKEDKRPRTAFTAEQLQRLKAEFQANRYITEQRRQTLAQELSLNESQIKIWFQNKRAKIKKATGIKNGLALHLMAQGLYNHSTTTVQDKDESE

SEQ ID NO: 3 - protein, 348 aa, Mus musculus
MSAAFPPSLMMMQRPLGSSTAFSIDSLIGSPPQPSPGHFVYTGYPMFMPYRPVVLPPPPPPPPALPQAALQPALPPAHPHHQIPSLPTGFCSSLAQGMALTSTLMATLPGGFSASPQHQEAAAARKFAPQPLPGGGNFDKAEALQADAEDGKAFLAKEGSLLAFSAAEAVQASLVGAVRGQGKDESKVEDDPKGKEESFSLESDVDYSSDDNLPGQTAHKEEDPGHALEETPQSGGAAGSTTSTGKNRRRRTAFTSEQLLELEKEFHCKKYLSLTERSQIAHALKLSEVQVKIWFQNRRAKWKRVKAGNANSKTGEPSRNPKIVVPIPVHVSRFAIRSQHQQLEQARP

SEQ ID NO: 4 - protein, 397 aa, Mus musculus
MEIVGCRAENNSCPFRPPAMLFHGISGGHIQGIMEEMERRSKTEARLTKGTQLNGRDAGMPPLSPEKPALCAGCGGKISDRYYLLAVDKQWHLRCLKCCECKLALESELTCFAKDGSIYCKEDYYRRFSVQRCARCHLGISASEMVMRARDSVYHLSCFTCSTCNKTLTTGDHFGMKDSLVYCRAHFETLLQGEYPPQLSYTELAAKSGGLALPYFNGTGTVQKGRPRKRKSPALGVDIVNYNSGCNENEADHLDRDQQPYPPSQKTKRMRTSFKHHQLRTMKSYFAINHNPDAKDLKQLAQKTGLTKRVLQVWFQNARAKFRRNLLRQENGGVDKADGTSLPAPPSADSGALTPPGTATTLTDLTNPTVTVVTTVTSNMDSHEPGSPSQTTLTNLF

SEQ ID NO: 5 - DNA, 20 bp, artificial sequence
  synthetic oligonucleotide
tggctcctggtacatcgaga

SEQ ID NO: 6 - DNA, 20 bp, artificial sequence
  Synthetic oligonucleotide
agcattggcaaccctgagaa

SEQ ID NO: 7 - DNA, 17 bp, artificial sequence
  Synthetic oligonucleotide
gggcctgctcaggctgt

SEQ ID NO: 8 - DNA, 20 bp, artificial sequence
  Synthetic oligonucleotide
gttctctgtgggggatcctg

SEQ ID NO: 9 - DNA, 20 bp, artificial sequence
  Synthetic oligonucleotide
ctcgctgcatcaggaagacc

SEQ ID NO: 10 - DNA, 19 bp, artificial sequence
  Synthetic oligonucleotide
taagaggagcaacccgtcg

SEQ ID NO: 11 - DNA, 21 bp, artificial sequence
  Synthetic oligonucleotide
gccagactataagccctaccc

SEQ ID NO: 12 - DNA, 20 bp, artificial sequence
  Synthetic oligonucleotide
gctgcacagggttacacttc

SEQ ID NO: 13 - DNA, 20 bp, artificial sequence
  Synthetic oligonucleotide
ccggtggtcaagactgactc

SEQ ID NO: 14 - DNA, 18 bp, artificial sequence
  Synthetic oligonucleotide
ctggtgcgtggaccagag

SEQ ID NO: 15 - DNA, 20 bp, artificial sequence
  Synthetic oligonucleotide
ccttcttcaggtcccaggtc

SEQ ID NO: 16 - DNA, 20 bp, artificial sequence
  Synthetic oligonucleotide
aactcagccttgagcctctg

SEQ ID NO: 17 - DNA, 19 bp, artificial sequence
  Synthetic oligonucleotide
attcctcttcgccgccatt

SEQ ID NO: 18 - DNA, 20 bp, artificial sequence
  Synthetic oligonucleotide
gaggcatcgatggccacttt

SEQ ID NO: 19 - DNA, 22 bp, artificial sequence
  Synthetic oligonucleotide
tctctagaggaacgctgagacc

SEQ ID NO: 20 - DNA, 22 bp, artificial sequence
  Synthetic oligonucleotide
gtagggtagcctttgagggatt

SEQ ID NO: 21 - DNA, 20 bp, artificial sequence
  Synthetic oligonucleotide
cccacctgtcagacccaagt

SEQ ID NO: 22 - DNA, 23 bp, artificial sequence
  Synthetic oligonucleotide
agtcatagaccagccctgtagca

SEQ ID NO: 23 - DNA, 20 bp, artificial sequence
  Synthetic oligonucleotide
ctgggaactgccaaagcaac

SEQ ID NO: 24 - DNA, 20 bp, artificial sequence
  Synthetic oligonucleotide
cctccgtttacctttcgcca

SEQ ID NO: 25 - DNA, 23 bp, artificial sequence
  Synthetic oligonucleotide
aatcgacaaatgggacctaatga

SEQ ID NO: 26 - DNA, 25 bp, artificial sequence
  Synthetic oligonucleotide
gtaaagatcctttcccaatctgttg

SEQ ID NO: 27 - DNA, 20 bp, artificial sequence
  Synthetic oligonucleotide
ggtggaagacaaggaggaag

SEQ ID NO: 28 - DNA, 19 bp, artificial sequence
  Synthetic oligonucleotide
aggaggagaaaaagccgag

SEQ ID NO: 29 - DNA, 18 bp, artificial sequence
  Synthetic oligonucleotide
ggcccggaacatctcagg

SEQ ID NO: 30 - DNA, 21 bp, artificial sequence
  Synthetic oligonucleotide
aaatctgtcaggctggtctgc

SEQ ID NO: 31 - DNA, 20 bp, artificial sequence
  Synthetic oligonucleotide
ggcgtaaacgcttcgagatg

SEQ ID NO: 32 - DNA, 21 bp, artificial sequence
  Synthetic oligonucleotide
cttcaggtagctggagtgagc

SEQ ID NO: 33 - DNA, 20 bp, artificial sequence
  Synthetic oligonucleotide
gaccccagcttgaagagtcc

SEQ ID NO: 34 - DNA, 20 bp, artificial sequence
  Synthetic oligonucleotide
ctgcccatccagttcgagtt

SEQ ID NO: 35 - DNA, 20 bp, artificial sequence
  Synthetic oligonucleotide
ctatccggatgttcgcctcc

SEQ ID NO: 36 - DNA, 20 bp, artificial sequence
  Synthetic oligonucleotide
gaggtgacctatctgggggt

SEQ ID NO: 37 - DNA, 20 bp, artificial sequence
  Synthetic oligonucleotide
atagcagcagtgagtccagc

SEQ ID NO: 38 - DNA, 23 bp, artificial sequence
  Synthetic oligonucleotide
gctggctaattttctgggtttca

SEQ ID NO: 39 - DNA, 20 bp, artificial sequence
  Synthetic oligonucleotide
cacagcacttgcaggaaagg

SEQ ID NO: 40 - DNA, 20 bp, artificial sequence
  Synthetic oligonucleotide
cctgtctgggtgtgtcgatt

SEQ ID NO: 41 - DNA, 22 bp, artificial sequence
  Synthetic oligonucleotide
cgtgtaagacattcctatctcg

SEQ ID NO: 42 - DNA, 21 bp, artificial sequence
  Synthetic oligonucleotide
gcccgctggcagaacgagaag

SEQ ID NO: 43 - DNA, 20 bp, artificial sequence
  Synthetic oligonucleotide
tactgcttagtggccagcct

SEQ ID NO: 44 - DNA, 20 bp, artificial sequence
  Synthetic oligonucleotide
aggcatttgcttgcacacac

SEQ ID NO: 45 - DNA, 22 bp, artificial sequence
  Synthetic oligonucleotide
gtactggacagtcctcacacca

SEQ ID NO: 46 - DNA, 22 bp, artificial sequence
  Synthetic oligonucleotide
ggtggtaccctatgcatttagc

SEQ ID NO: 47 - DNA, 20 bp, artificial sequence
  Synthetic oligonucleotide
agaggtcaagaagggcaagc

SEQ ID NO: 48 - DNA, 20 bp, artificial sequence
  Synthetic oligonucleotide
tgccactcaacgctctttct

SEQ ID NO: 49 - DNA, 20 bp, artificial sequence
  Synthetic oligonucleotide
gcgtggccagtgtaaaagca

SEQ ID NO: 50 - DNA, 21 bp, artificial sequence
  Synthetic oligonucleotide
cgcattcttcacagatggtgt